European Patent Specification EP 3 464 379 B1, published September 27, 2023. Title: Antibodies, uses thereof and conjugates thereof. Applicant: Polytherics Limited. The sequence listing filed with the application follows.

SEQUENCE LISTING (38 sequences)

SEQ ID NO: 1 - DNA, 345 bp, Artificial Sequence
  synthetic construct
gaggtccagctggtgcagtctggacctgagctgaagaagcctggggcctcagtgaaggtctcctgcaagacttctggatacacattcactgaatacaccatccactgggtgaagcaggcccatggaaagggccttgagtggattggaaacattaatcctaacaatggtggtactacctacaaccagaagttcgaggacagagccacattgactgtagacaagtccaccagcacagcctacatggagctcagcagcctgagatctgaggatactgcagtctattactgtgcagctggttggaactttgactactggggccaaggcaccacggtcaccgtctcctca

SEQ ID NO: 2 - DNA, 345 bp, Artificial Sequence
  synthetic construct
gaggtccagctggtgcagtctggagctgaggtgaagaagcctggggcctcagtgaaggtctcctgcaagacttctggatacacattcactgaatacaccatccactgggtgaagcaggcccctggaaagggccttgagtggattggaaacattaatcctaacaatggtggtactacctacaaccagaagttcgaggacagagccacaatcactgtagacaagtccaccagcacagcctacatggagctcagcagcctgagatctgaggatactgcagtctattactgtgcagctggttggaactttgactactggggccaaggcaccacggtcaccgtctcctca

SEQ ID NO: 3 - DNA, 345 bp, Artificial Sequence
  synthetic construct
gaggtccagctggtgcagtctggagctgaggtgaagaagcctggggcctcagtgaaggtctcctgcaagacttctggatacacattcactgaatacaccatccactgggtgaggcaggcccctggaaagggccttgagtggattggaaacattaatcctaacaatggtggtactacctacaaccagaagttcgaggacagagccacaatcactgtagacaagtccaccagcacagcctacatggagctcagcagcctgagatctgaggatactgcagtctattactgtgcagctggttggaactttgactactggggccaaggcaccacggtcaccgtctcctca

SEQ ID NO: 4 - DNA, 345 bp, Artificial Sequence
  synthetic construct
gaggtccagctggtgcagtctggagctgaggtgaagaagcctggggcctcagtgaaggtctcctgcaaggcttctggatacacattcactgaatacaccatccactgggtgaggcaggcccctggaaagggccttgagtggattggaaacattaatcctaacaatggtggtactacctacaaccagaagttcgaggacagagtcacaatcactgtagacaagtccaccagcacagcctacatggagctcagcagcctgagatctgaggatactgcagtctattactgtgcagctggttggaactttgactactggggccaaggcaccacggtcaccgtctcctca

SEQ ID NO: 5 - DNA, 345 bp, Artificial Sequence
  synthetic construct
gaggtccagctggtgcagtctggagctgaggtgaagaagcctggggcctcagtgaaggtctcctgcaaggcttctggatacacattcactgaatacaccatccactgggtgaggcaggcccctggaaagggccttgagtggattggaaacattaatcctaaccagggtggtactacctacaaccagaagttcgaggacagagtcacaatcactgtagacaagtccaccagcacagcctacatggagctcagcagcctgagatctgaggatactgcagtctattactgtgcagctggttggaactttgactactggggccaaggcaccacggtcaccgtctcctca

SEQ ID NO: 6 - DNA, 321 bp, Artificial Sequence
  synthetic construct
gacattgtgatgacccagtctcccagcttcctgtccgcatcagtaggagacagggtcaccatcacttgcaaggccagtcaggatgtgggtactgctgtagactggtatcaacagaaaccagggcaagctcctaaactactgatttactgggcatccacccggcacactggagtccctgatcgcttcacaggcagtggatctgggacagatttcactctcaccatcagcagactgcagtctgaagactttgcagattatttctgtcagcaatataacagctatcctctcacgttcggccaggggaccatggtggatatcaaa

SEQ ID NO: 7 - DNA, 321 bp, Artificial Sequence
  synthetic construct
gacattgtgatgacccagtctcccagcaccctgtccgcatcagtaggagacagggtcaccatcacttgcaaggccagtcaggatgtgggtactgctgtagactggtatcaacagaaaccagggcaagctcctaaactactgatttactgggcatccacccggcacactggagtccctgatcgcttcacaggcagtggatctgggacagatttcactctcaccatcagcagactgcagtctgaagactttgcagattatttctgtcagcaatataacagctatcctctcacgttcggccaggggaccaaggtggatatcaaa

SEQ ID NO: 8 - DNA, 321 bp, Artificial Sequence
  synthetic construct
gacattgtgatgacccagtctcccagcaccctgtccgcatcagtaggagacagggtcaccatcacttgcaaggccagtcaggatgtgggtactgctgtagactggtatcaacagaaaccagggcaagctcctaaactactgatttactgggcatccacccggcacactggagtccctgatcgcttcagcggcagtggatctgggacagatttcactctcaccatcagcagactgcagcctgaagactttgcagattattactgtcagcaatataacagctatcctctcacgttcggccaggggaccaaggtggatatcaaa

SEQ ID NO: 9 - DNA, 321 bp, Artificial Sequence
  synthetic construct
gacattcagatgacccagtctcccagcaccctgtccgcatcagtaggagacagggtcaccatcacttgcaaggccagtcaggatgtgggtactgctgtagactggtatcaacagaaaccagggcaagctcctaaactactgatttactgggcatccacccggcacactggagtccctgatcgcttcagcggcagtggatctgggacagatttcactctcaccatcagcagactgcagcctgaagactttgcagtttattactgtcagcaatataacagctatcctctcacgttcggccaggggaccaaggtggatatcaaa

SEQ ID NO: 10 - protein, 115 aa, Artificial Sequence
  synthetic construct
EVQLVQSGPELKKPGASVKVSCKTSGYTFTEYTIHWVKQAHGKGLEWIGNINPNNGGTTYNQKFEDRATLTVDKSTSTAYMELSSLRSEDTAVYYCAAGWNFDYWGQGTTVTVSS

SEQ ID NO: 11 - protein, 115 aa, Artificial Sequence
  synthetic construct
EVQLVQSGAEVKKPGASVKVSCKTSGYTFTEYTIHWVKQAPGKGLEWIGNINPNNGGTTYNQKFEDRATITVDKSTSTAYMELSSLRSEDTAVYYCAAGWNFDYWGQGTTVTVSS

SEQ ID NO: 12 - protein, 115 aa, Artificial Sequence
  synthetic construct
EVQLVQSGAEVKKPGASVKVSCKTSGYTFTEYTIHWVRQAPGKGLEWIGNINPNNGGTTYNQKFEDRATITVDKSTSTAYMELSSLRSEDTAVYYCAAGWNFDYWGQGTTVTVSS

SEQ ID NO: 13 - protein, 115 aa, Artificial Sequence
  synthetic construct
EVQLVQSGAEVKKPGASVKVSCKASGYTFTEYTIHWVRQAPGKGLEWIGNINPNNGGTTYNQKFEDRVTITVDKSTSTAYMELSSLRSEDTAVYYCAAGWNFDYWGQGTTVTVSS

SEQ ID NO: 14 - protein, 115 aa, Artificial Sequence
  synthetic construct
EVQLVQSGAEVKKPGASVKVSCKASGYTFTEYTIHWVRQAPGKGLEWIGNINPNQGGTTYNQKFEDRVTITVDKSTSTAYMELSSLRSEDTAVYYCAAGWNFDYWGQGTTVTVSS

SEQ ID NO: 15 - protein, 107 aa, Artificial Sequence
  synthetic construct
DIVMTQSPSFLSASVGDRVTITCKASQDVGTAVDWYQQKPGQAPKLLIYWASTRHTGVPDRFTGSGSGTDFTLTISRLQSEDFADYFCQQYNSYPLTFGQGTMVDIK

SEQ ID NO: 16 - protein, 107 aa, Artificial Sequence
  synthetic construct
DIVMTQSPSTLSASVGDRVTITCKASQDVGTAVDWYQQKPGQAPKLLIYWASTRHTGVPDRFTGSGSGTDFTLTISRLQSEDFADYFCQQYNSYPLTFGQGTKVDIK

SEQ ID NO: 17 - protein, 107 aa, Artificial Sequence
  synthetic construct
DIVMTQSPSTLSASVGDRVTITCKASQDVGTAVDWYQQKPGQAPKLLIYWASTRHTGVPDRFSGSGSGTDFTLTISRLQPEDFADYYCQQYNSYPLTFGQGTKVDIK

SEQ ID NO: 18 - protein, 107 aa, Artificial Sequence
  synthetic construct
DIQMTQSPSTLSASVGDRVTITCKASQDVGTAVDWYQQKPGQAPKLLIYWASTRHTGVPDRFSGSGSGTDFTLTISRLQPEDFAVYYCQQYNSYPLTFGQGTKVDIK

SEQ ID NO: 19 - DNA, 345 bp, Artificial Sequence
  synthetic construct
gaggtccagctgcaacagtctggacctgagctgaagaagcctgggacttcagtgaggatatcctgcaagacttctggatacacattcactgaatacaccatccactgggtgaagcagagccatggaaagagccttgagtggattggaaacattaatcctaacaatggtggtactacctacaaccagaagttcgaggacaaggccacattgactgtagacaagtcctccagcacagcctacatggagctccgcagcctgacatctgaggattctgcagtctattactgtgcagctggttggaactttgactactggggccaaggcaccacgctcaccgtctcctca

SEQ ID NO: 20 - DNA, 321 bp, Artificial Sequence
  synthetic construct
gacattgtgatgacccagtctcacaaattcatgtccacatcagtaggagacagggtcagcatcatctgcaaggccagtcaggatgtgggtactgctgtagactggtatcaacagaaaccagggcaatctcctaaactactgatttactgggcatccacccggcacactggagtccctgatcgcttcacaggcagtggatctgggacagatttcactctcaccatcaccaatgtgcagtctgaagacctggcagattatttctgtcagcaatataacagctatcctctcacgttcggcgccgggaccatgctggatctcaaa

SEQ ID NO: 21 - DNA, 345 bp, Artificial Sequence
  synthetic construct
gaggtccaactggtacagtctggacctgaagtgaagaagcctggggctacagtgaagatatcctgcaagacttctggatacacattcactgaatataccatacactgggtgaagcaggcccctggaaagggccttgagtggattggaaacatcaatcctaacaatggtggtaccacctacaatcagaagttcgaggacaaggccacactaactgtagacaagtccaccgatacagcctacatggagctcagcagcctaagatctgaggatactgcagtctattattgtgcagctggttggaactttgactactggggccaagggaccctgctcaccgtctcctca

SEQ ID NO: 22 - DNA, 321 bp, Artificial Sequence
  synthetic construct
gacatccagatgacccagtctccctcatccctgtccacatcagtaggagacagggtcaccctcacctgtaaggccagtcaagatgtgggtactgctgtagactggtatcaacagaaaccaggaccatctcctaaactactgatttattgggcatccactcggcacactggaatccctagtcgcttctcaggcagtggatctgggacagacttcactctcaccatttctagtcttcagcctgaagactttgcagattattactgtcagcaatataacagctatcctctcacgttcggtcctgggaccaaggtggacatcaaa

SEQ ID NO: 23 - protein, 115 aa, Artificial Sequence
  synthetic construct
EVQLQQSGPELKKPGTSVRISCKTSGYTFTEYTIHWVKQSHGKSLEWIGNINPNNGGTTYNQKFEDKATLTVDKSSSTAYMELRSLTSEDSAVYYCAAGWNFDYWGQGTTLTVSS

SEQ ID NO: 24 - protein, 107 aa, Artificial Sequence
  synthetic construct
DIVMTQSHKFMSTSVGDRVSIICKASQDVGTAVDWYQQKPGQSPKLLIYWASTRHTGVPDRFTGSGSGTDFTLTITNVQSEDLADYFCQQYNSYPLTFGAGTMLDLK

SEQ ID NO: 25 - protein, 115 aa, Artificial Sequence
  synthetic construct
EVQLVQSGPEVKKPGATVKISCKTSGYTFTEYTIHWVKQAPGKGLEWIGNINPNNGGTTYNQKFEDKATLTVDKSTDTAYMELSSLRSEDTAVYYCAAGWNFDYWGQGTLLTVSS

SEQ ID NO: 26 - protein, 107 aa, Artificial Sequence
  synthetic construct
DIQMTQSPSSLSTSVGDRVTLTCKASQDVGTAVDWYQQKPGPSPKLLIYWASTRHTGIPSRFSGSGSGTDFTLTISSLQPEDFADYYCQQYNSYPLTFGPGTKVDIK

SEQ ID NO: 27 - DNA, 348 bp, Artificial Sequence
  synthetic construct
gaagtgaaacttgaggagtctggaggaggcttggtgcaacctggagggtccatgaaaatctcctgtgttgcctctggattcactttcagtaattactggatgaactgggtccgccagtctccagagaaggggcttgagtgggttgctgaaattagatcgcaatctaataattttgcaacacattatgcggagtctgtgaaagggagggtcatcatctcaagagatgattccaagagtagtgtctacctgcaaatgaacagtttgagagctgaagacactgccgtttattactgtaccaggcgatggaataatttctggggccaaggcaccactgtcacagtctcctca

SEQ ID NO: 28 - DNA, 321 bp, Artificial Sequence
  synthetic construct
aacattgtaatgacccaatttcccaaatccatgtccgcctcagcaggagagaggatgaccttgacctgcaaggccagtgagaatgtgggtacttatgtgtcctggtatcaacagaaaccaacacagtctcctaagatgttgatatacggggcatccaaccggttcactggggtcccagatcgcttctccggcagtggatctggaacagatttcattctgaccatcagcagtgtgcaggcagaagaccttgtagattattactgtggacagagttacacctttccgtacacgttcggaggggggaccaagctggaaatgaag

SEQ ID NO: 29 - protein, 116 aa, Artificial Sequence
  synthetic construct
EVKLEESGGGLVQPGGSMKISCVASGFTFSNYWMNWVRQSPEKGLEWVAEIRSQSNNFATHYAESVKGRVIISRDDSKSSVYLQMNSLRAEDTAVYYCTRRWNNFWGQGTTVTVSS

SEQ ID NO: 30 - protein, 107 aa, Artificial Sequence
  synthetic construct
NIVMTQFPKSMSASAGERMTLTCKASENVGTYVSWYQQKPTQSPKMLIYGASNRFTGVPDRFSGSGSGTDFILTISSVQAEDLVDYYCGQSYTFPYTFGGGTKLEMK

SEQ ID NO: 31 - DNA, 2253 bp, Artificial Sequence
  synthetic construct
atgtggaacctgctgcacgagacagacagcgccgtggccaccgccagacggcctagatggctgtgtgccggcgctctggtgctggctggcggcttcttcctgctgggcttcctgttcggctggttcatcaagagcagcaacgaggccaccaacatcacccccaagcacaacatgaaggcctttctggacgagctgaaggccgagaatatcaagaagttcctgtacaacttcacccagatcccccacctggccggcaccgagcagaacttccagctcgccaagcagatccagagccagtggaaagagttcggcctggacagcgtggaactggcccactacgacgtgctgctgagctaccccaacaagacccaccccaactacatcagcatcatcaacgaggacggcaacgagattttcaacaccagcctgttcgagccccctccacccggctacgagaacgtgtccgacatcgtgcccccattcagcgccttcagtccacaaggcatgcccgagggcgacctggtgtacgtgaactacgcccggaccgaggacttcttcaagctggaacgggacatgaagatcaactgctccggcaagatcgtgatcgccagatacggcaaggtgttccggggcaacaaagtgaagaacgcccagctcgctggggccaagggcgtgatcctgtacagcgaccccgccgactacttcgcccctggcgtgaagtcctaccccgacggctggaatctgcctggcggcggagtgcagcggggcaacatcctgaacctgaacggcgctggcgaccccctgacacctggctaccccgccaacgagtacgcctacagacggggaatcgccgaggccgtgggcctgcctagcatccctgtgcaccccatcggctactacgacgcccagaaactgctggaaaagatgggcggcagcgcccctcccgacagctcttggagaggcagcctgaaggtgccctacaacgtgggccctggcttcaccggcaacttcagcacccagaaagtgaagatgcacatccacagcaccaacgaagtgacccggatctacaacgtgatcggcaccctgagaggcgccgtggaacccgacagatacgtgatcctgggcggccaccgggatagctgggtgttcggcggcatcgaccctcagtctggcgccgctgtggtgcacgagatcgtgcggagctttggcaccctgaagaaagagggctggcggcccagacggaccatcctgttcgcctcttgggacgccgaggaattcggcctgctgggcagcaccgagtgggccgaggaaaacagcagactgctccaggaacggggcgtcgcctacatcaacgccgacagcagcatcgagggcaactacaccctgcgggtggactgcacccccctgatgtacagcctggtgcacaacctgaccaaagagctgaagtcccccgacgagggcttcgagggcaagagcctgtacgagagctggaccaagaagtcccccagccccgagttcagcggcatgcccagaatcagcaagctgggcagcggcaacgacttcgaggtgttcttccagcggctgggaatcgccagcggcagagcccggtacaccaagaactgggagacaaacaagttctccggctaccccctgtaccacagcgtgtacgagacatacgagctggtggaaaagttctacgaccccatgttcaagtaccacctgaccgtggcccaagtgcgcggaggcatggtgttcgagctggccaacagcatcgtgctgcccttcgactgccgggactacgccgtggtgctgcggaagtacgccgacaaaatctacagcatcagcatgaagcacccccaggaaatgaagacctacagcgtgtccttcgacagcctgttcagcgccgtgaagaatttcaccgagatcgccagcaagttcagcgagcggctccaggacttcgacaagagcaaccccatcgtgctgagaatgatgaacgaccagctcatgttcctggaacgggccttcatcgaccccctgggcctgcccgaccggcccttctacagacacgtgatctatgcccccagcagccacaacaaatacgccggcgagagcttccccggaatctacgatgccctgttcgacatcgagagcaaggtggaccccagcaaggcctggggcgaagtgaagcggcaaatctacgtggccgccttcacagtgcaagccgctgccgagacactgagcgaagtggcctag

SEQ ID NO: 32 - protein, 750 aa, Artificial Sequence
  synthetic construct
MWNLLHETDSAVATARRPRWLCAGALVLAGGFFLLGFLFGWFIKSSNEATNITPKHNMKAFLDELKAENIKKFLYNFTQIPHLAGTEQNFQLAKQIQSQWKEFGLDSVELAHYDVLLSYPNKTHPNYISIINEDGNEIFNTSLFEPPPPGYENVSDIVPPFSAFSPQGMPEGDLVYVNYARTEDFFKLERDMKINCSGKIVIARYGKVFRGNKVKNAQLAGAKGVILYSDPADYFAPGVKSYPDGWNLPGGGVQRGNILNLNGAGDPLTPGYPANEYAYRRGIAEAVGLPSIPVHPIGYYDAQKLLEKMGGSAPPDSSWRGSLKVPYNVGPGFTGNFSTQKVKMHIHSTNEVTRIYNVIGTLRGAVEPDRYVILGGHRDSWVFGGIDPQSGAAVVHEIVRSFGTLKKEGWRPRRTILFASWDAEEFGLLGSTEWAEENSRLLQERGVAYINADSSIEGNYTLRVDCTPLMYSLVHNLTKELKSPDEGFEGKSLYESWTKKSPSPEFSGMPRISKLGSGNDFEVFFQRLGIASGRARYTKNWETNKFSGYPLYHSVYETYELVEKFYDPMFKYHLTVAQVRGGMVFELANSIVLPFDCRDYAVVLRKYADKIYSISMKHPQEMKTYSVSFDSLFSAVKNFTEIASKFSERLQDFDKSNPIVLRMMNDQLMFLERAFIDPLGLPDRPFYRHVIYAPSSHNKYAGESFPGIYDALFDIESKVDPSKAWGEVKRQIYVAAFTVQAAAETLSEVA

SEQ ID NO: 33 - protein, 115 aa, Artificial Sequence; identical to SEQ ID NO: 13
  synthetic construct
  VARIANT (9)..(9): The residue at this position may be Ala or Pro
  VARIANT (11)..(11): The residue at this position may be Val or Leu
  VARIANT (24)..(24): The residue at this position may be Ala or Thr
  VARIANT (38)..(38): The residue at this position may be Arg or Lys
  VARIANT (41)..(41): The residue at this position may be Pro or His
  VARIANT (55)..(55): The residue at this position may be Asn or Gln
  VARIANT (68)..(68): The residue at this position may be Val or Ala
  VARIANT (70)..(70): The residue at this position may be Ile or Leu

SEQ ID NO: 34 - protein, 107 aa, Artificial Sequence; identical to SEQ ID NO: 18
  synthetic construct
  VARIANT (3)..(3): The residue at this position may be Gln or Val
  VARIANT (10)..(10): The residue at this position may be Thr or Phe
  VARIANT (63)..(63): The residue at this position may be Ser or Thr
  VARIANT (80)..(80): The residue at this position may be Pro or Ser
  VARIANT (85)..(85): The residue at this position may be Val or Asp
  VARIANT (87)..(87): The residue at this position may be Tyr or Phe
  VARIANT (103)..(103): The residue at this position may be Lys or Met

SEQ ID NO: 35 - protein, 142 aa, Artificial Sequence
  synthetic construct
MELGLRWGFLVALLRGVQCQVQLVESGGGVVQPGRSLRLSCAASGFAFSRYGMHWVRQAPGKGLEWVAVIWYDGSNKYYADSVKGRFTISRDNSKNTQYLQMNSLRAEDTAVYYCARGGDFLYYYYYGMDVWGQGTTVTVSS

SEQ ID NO: 36 - protein, 127 aa, Artificial Sequence
  synthetic construct
MRVPAQLLGLLLLWLPDTRCDIQMTQSPSSLSASVGDRVTITCRASQGISNYLAWYQQKTGKVPKFLIYEASTLQSGVPSRFSGGGSGTDFTLTISSLQPEDVATYYCQNYNSAPFTFGPGTKVDIK

SEQ ID NO: 37 - protein, 143 aa, Artificial Sequence
  synthetic construct
MELGLRWVLLVALLRGVQCQVQLVESGGGVVQPGRSLRLSCAASGFTFSNYVMHWVRQAPGKGLEWVAIIWYDGSNKYYADSVKGRFTISRDNSKNTLYLQMNSLRAEDTAVYYCAGGYNWNYEYHYYGMDVWGQGTTVTVSS

SEQ ID NO: 38 - protein, 127 aa, Artificial Sequence
  synthetic construct
MRVPAQLLGLLLLCFPGARCDIQMTQSPSSLSASVGDRVTITCRASQGITNYLAWFQQKPGKAPKSLIYAASSLQSGVPSKFSGSGSGTDFSLTISSLQPEDFATYYCQQYNSYPITFGQGTRLEIK